European Patent Application EP 4 310 100 A1, published January 24, 2024. Title: A monoclonal antibody specifically binding to a sugar chain in which a terminal sialic acid residue is bound to galactose with an  ¿2,6 bond, and a method for measuring a sugar chain in which a terminal sialic acid residue is bound to galactose with an  ¿2,6 bond. Applicant: HIROSAKI UNIVERSITY SYSTEM INSTRUMENTS Co., Ltd. The sequence listing filed with the application follows.

SEQUENCE LISTING (16 sequences)

SEQ ID NO: 1 - protein, 8 aa, Oryctolagus cuniculus
ASGFSFSN

SEQ ID NO: 2 - protein, 8 aa, Oryctolagus cuniculus
CIVTRDSN

SEQ ID NO: 3 - protein, 11 aa, Oryctolagus cuniculus
CARVVNGSFRL

SEQ ID NO: 4 - protein, 8 aa, Oryctolagus cuniculus
QSVYNKNW

SEQ ID NO: 5 - protein, 3 aa, Oryctolagus cuniculus
AAS

SEQ ID NO: 6 - protein, 10 aa, Oryctolagus cuniculus
QGDFSGNIHS

SEQ ID NO: 7 - protein, 8 aa, Oryctolagus cuniculus
ASGFSFSG

SEQ ID NO: 8 - protein, 7 aa, Oryctolagus cuniculus
CFWFSSG

SEQ ID NO: 9 - protein, 11 aa, Oryctolagus cuniculus
CARRGDNTYGL

SEQ ID NO: 10 - protein, 6 aa, Oryctolagus cuniculus
QSISSY

SEQ ID NO: 11 - protein, 3 aa, Oryctolagus cuniculus
YAS

SEQ ID NO: 12 - protein, 12 aa, Oryctolagus cuniculus
QNTARSSNNGDP

SEQ ID NO: 13 - protein, 116 aa, Oryctolagus cuniculus
QSLEESGGDLVKPGASLTLTCTASGFSFSNNYWICWVRQAPGKGLEWIGCIVTRDSNTAYANWAKGRLTISKTSSTTVTLQMTSLTVADTATYFCARVVNGSFRLWGPGTLVTVSS

SEQ ID NO: 14 - protein, 110 aa, Oryctolagus cuniculus
AQVLTQTASPVSAPVGGTVTINCQSSQSVYNKNWLSWYQQKPGQPPKLLINAASNLASGVPSRFSGSGSGTQFTLTISDLECDDAATYYCQGDFSGNIHSFGGGTEVVVK

SEQ ID NO: 15 - protein, 117 aa, Oryctolagus cuniculus
QEQLVESGGGLVQPEGSLTLTCTASGFSFSGIYAMCWVRQAPGKGLEWIACFWFSSGSTYYATWAKGRFTISKTSSTTVTLQMTSLTAADTATYFCARRGDNTYGLWGPGTLVTVSS

SEQ ID NO: 16 - protein, 110 aa, Oryctolagus cuniculus
ALVMTQTPASVSAAVGGTVTIKCQASQSISSYCSWYQQKPGQRPKLLIYYASKLASGVPSRFKGSGSGTEFTLTISDLECADAATYYCQNTARSSNNGDPFGGGTEVVVK